European Patent Specification EP 3 197 270 B1, published December 3, 2025. Title: Wheat Ms1 Polynucleotides, Polypeptides, and Methods of Use. Applicant: Pioneer Hi-Bred International, Inc. The sequence listing filed with the application follows.

SEQUENCE LISTING (47 sequences)

SEQ ID NO: 1 - DNA, 3838 bp, Hordeum vulgare
  promoter (1)..(902)
cgcacatcaacataaactcatcagatgggaataatcggatctacgaaggacataaaactctttaatctcatgacaacgccagaagagcaagagtaaatatattctcataaaaaacaatgaacactagatgatgacgaagaacataagattcttcaaggagaaattgcggcagcggagatggcagccggaggcgagggggccaaaaactctgttgcggcggcagcggtagccttggtgaaacccacacgtttgcacaccatataagttgtttgcaagggttacatgggcctcgctctcgtgaaaaagaaggtcatacatgggtcttggtctcgtgcaaaacgaaaggtcagcagtccatgggccggaggaaaaaccgggcaacaacacgccatgtgtgttttcgcgggaacccaattccgaaatcactcaccggcacctcgtcccgatgccttccagaacgttctacgtgcttccacagggccagcccagccgtgggatcagatcaggatcagcacgaacattgaagctagcgcggcgatatttttcccagcctccgcctcgctcgacgactgcatttcatttcgaaaacaaaaaaaagagctttctccttctcatcccgagcgccagaggagcaccagaaaggccacccacccaccctcacgtaccgccctcgcacccgcgcggccacatctgggccgtccacttgggcagctggccgttccattcccgaactgacgggcaggatcgagcgagcggcgcgcccacggctcctccggctatataacccgccacccacaccactcccctccggcgttccaccagagccttcctccctccaccgcaccaccaccaccaccgcgccaaaaaccctagggagcgagcgagctcacctcgccccgcccatggagagatcccgccgcctgctgctcgtggcggggctcctcgccgcgctgctcccggcggcggccgccaccttcgggctgcagcagggggcgcagtgcgaccccacgttcctggcgacgcaggccgcgctcttctgcgcccccgacatgcccacggcccagtgctgcgagcccgtcgtcgccgccttcgacctcgggggcggcgtcccctgcctctgccgcgtcgccgccgagccgcagctggtcatggcggggctcaacgccacccacctcttcgcgctgtacacctcctgcggcggcatccgtcccggtggcgcccacctcgccgccgcctgccaaggtacgttcacgttcaccgcctccctccctctccttctctctttgcacctgtaccagccgattcggcgttcgctttcgcgtttcccggtagttttgatggtttctcgagtcgccagtgctccgatttgggttcggtttccttgcgttgtaccggatctgcctgtacggcgcgcggcgtcggggttctcgttgtttcccgtggcgagcatccccgcgcgcccacggcctagctagcttaccttcagatacgcggagcgatttaggatcagtatgaggagttcgtcgtagaagaatgcatgcggaacgcgcgattgtttgtttcatcgattttggatctgtgataggcctgcttgttcccgagtttttgcacgtagaagaatcatgtgcagaacccctggtccattatttgttatgtatatacacgattacttgtgcatatgcagaagtcttagttatctgctacccttccagaattattcgtggtgtttttgttcctctagttaaacttcagatgatctttcgttcgagtttattttcctgcctgtaactgagatcgatatacctatcaccgtgactgtgagagagacagagagttgttgccgtttaactgctatatatatgtacgttttctgctactgtttaatcgactgctccatcccgttcgcgataggacttgtttcaaaccgtcacgcagctctgcttcctgcagtgtcttttgtcttcgtttggtcaaaactgaaaacgcttgctatcgaggccagaggcagggcaaaagctccccgtacttttcgctttgcagtggcatctctttctttttttttgccgaaaattgtttccacgttcatccccgggtgtcgtactacttaattatctgcatgcagttttcgtgtccttcctccgtcgtgaaaaaaaggttgggtcaaatgaatcaaccgtgtatgcagggcagcagcaacagagatagagtagctggctgtcgcagctttaacaaaagcagtctgtggcctgccacagttttcctgatttttgtttaatctggcctgggcttcttttcttgttgcgcacgtcgtcgcctccttcttttttcccaattttttgatttcttttgagataaggacacgaacggctggtaactgacttttcttgttgttttttactgtgggttttggacgcaggaccggctcccccggccgccgtcgtcagcagccccccgccaccatcgccagcacctcgccgcaaacaggcagcgcgtacgaacctctcgctctctctctctccctctcgcctgcatctcgctctgtacataacctattgggttcatatgctgatcagcgttgacatactaacttgttcatttgattctcagacgacgcgcctccaccgccgccgtccagcgagaagccatccccgccgccccaggagcatgacggcgccgcacacgccaagagcgcccccgccctcgcggctcctaccccgctcgcgcccgctgccgctactgccccgccgcccgaggcgccacactccgccgcgtcgtcgtccgattcggccttcatcttcatcgccgcggccatgctcgccatttacatcgtcctctgaatggccgacccccaaggcagcagagtacttgtcatctgattccgtttcatgcttgtcgccgtttgttgaggttcgtttctgcagtccgaacaagacggtggggttttgatcgggtacccagatttctatgtcgatcgcgcgtactagtactagtagttgcttagcagatgaacgaacattgggttttgggattcctctagctgatgaaccactgctattttccatgtgatcgatggatatgatctgaatggatggatgaagttttggtttctgatgctgatgatgtgctgcttcttcatttgcatgctcgatctattccttcaattttgtggagcaacagtttgtttagcttctgttctgctatgaataatgccgcttgcatcttgtcattgctgataatctgcttaatgcagacattgcttccgtcccaaacaatctgttgcttaccaggtaatgcatataatctgtacctcaccttcgcacaacaacagaagctaccctgctaaaaaaacacacacacacacacaaaaaaaacagaagctggtctcacacggaagccgcttcggggactgtttgcagctttttattgccattttgtttttcatgcaggtacaaatcgagggtgttgcttgatttgatcatggatgatcacttagagcaacatgtgtgttttgtctgtgttttattcgttgctcgtccatccaatttaaacttgaaatggatcgtgtgtggataaaagaagacgtgcgtcagtttgaatcgacgcgttgggttatattttgtgtctgtgacgaccgaaacgaagacaaaatatatcgtccggttagaattgctctaatgctagctttctctcctaccatcgcattccgtggtaggaaaaagtactagaaccacaggaaactggaacgcaagaaaagcatatctaccgttggccgttgatcttgtttcacattcggtatggctccggtcatattgttggagattcacattcatgcacgcaa

SEQ ID NO: 2 - DNA, 642 bp, Hordeum vulgare
atggagagatcccgccgcctgctgctcgtggcggggctcctcgccgcgctgctcccggcggcggccgccaccttcgggctgcagcagggggcgcagtgcgaccccacgttcctggcgacgcaggccgcgctcttctgcgcccccgacatgcccacggcccagtgctgcgagcccgtcgtcgccgccttcgacctcgggggcggcgtcccctgcctctgccgcgtcgccgccgagccgcagctggtcatggcggggctcaacgccacccacctcttcgcgctgtacacctcctgcggcggcatccgtcccggtggcgcccacctcgccgccgcctgccaaggaccggctcccccggccgccgtcgtcagcagccccccgccaccatcgccagcacctcgccgcaaacaggcagcgcacgacgcgcctccaccgccgccgtccagcgagaagccatccccgccgccccaggagcatgacggcgccgcacacgccaagagcgcccccgccctcgcggctcctaccccgctcgcgcccgctgccgctactgccccgccgcccgaggcgccacactccgccgcgtcgtcgtccgattcggccttcatcttcatcgccgcggccatgctcgccatttacatcgtcctc

SEQ ID NO: 3 - protein, 214 aa, Hordeum vulgare
MERSRRLLLVAGLLAALLPAAAATFGLQQGAQCDPTFLATQAALFCAPDMPTAQCCEPVVAAFDLGGGVPCLCRVAAEPQLVMAGLNATHLFALYTSCGGIRPGGAHLAAACQGPAPPAAVVSSPPPPSPAPRRKQAAHDAPPPPPSSEKPSPPPQEHDGAAHAKSAPALAAPTPLAPAAATAPPPEAPHSAASSSDSAFIFIAAAMLAIYIVL

SEQ ID NO: 4 - DNA, 660 bp, Triticum aestivum
atggagagatcccgcgggctgctgctggtggcggggctgctggcggcgctgctgccggcggcggcggcgcagccgggggcgccgtgcgagcccgcgctgctggcgacgcaggtggcgctcttctgcgcgcccgacatgccgacggcccagtgctgcgagcccgtcgtcgccgccgtcgacctcggcggcggggtgccctgcctctgccgcgtcgccgccgagccgcagctcgtcatggcgggcctcaacgccacccacctcctcacgctctacagctcctgcggcggcctccgccccggcggcgcccacctcgccgccgcctgcgaaggacccgctcccccggccgccgtcgtcagcagccccccgcccccgcctccaccgtccgccgcacctcgccgcaagcagccagcgcacgacgcaccaccgccgccaccgccgtcgagcgagaagccgtcgtccccgccgccgtcccaggaccacgacggcgccgccccccgcgccaaggccgcgcccgcccaggcggccacctccacgctcgcgcccgccgccgccgccaccgccccgccgccccaggcgccgcactccgccgcgcccacggcgccgtccaaggcggccttcttcttcgtcgccacggccatgctcggcctctacatcatcctc

SEQ ID NO: 5 - protein, 220 aa, Triticum aestivum
MERSRGLLLVAGLLAALLPAAAAQPGAPCEPALLATQVALFCAPDMPTAQCCEPVVAAVDLGGGVPCLCRVAAEPQLVMAGLNATHLLTLYSSCGGLRPGGAHLAAACEGPAPPAAVVSSPPPPPPPSAAPRRKQPAHDAPPPPPPSSEKPSSPPPSQDHDGAAPRAKAAPAQAATSTLAPAAAATAPPPQAPHSAAPTAPSKAAFFFVATAMLGLYIIL

SEQ ID NO: 6 - DNA, 1527 bp, Triticum aestivum
agacttaaaccatttagttacaaatatcgatgcacaccttcggtggggcgttgtgaaaaagcatgttttttgggtcgacaagccccttttgcaacgtatcctcttctaatcctattcagatcattaacatcataagctgcaattgacatgctcttctgaggatcaggttcatgcaattaaacatcataaactgcatctttgatgtcatccttttcctatattttttccagattattggcttgcttcgttttcaatatcaggttctatgattcgacttctgttgttgccagtaataatttgtagttgctgcggaatatgaactcaaggagagctgatggtgctatgaagttgatttgatgggaggttgttctacacctgcacttgctgctcgacttaaatacatgccttggatttcttcccagctctagtacataatatttttcaaattaatgttccacgacataaaatttaaatccacaaacatatttttagtacatgaacaattttctaatatagggcaaacatttttcatatacaaaccgatcattttaatatatggtgaaaatcagtgtaatatatgctgaaatgttttcaaatacatattgaacatatttataataaatggtgaacattttttttaataattgatgaccatttttaaaatgcatattgaacattttataatatacactgtacagttttataataatcgacgaacatcttttggagttctgaacatttttttcaaaaacacaagccattttccaggaagaatacaaatgcaaaagaaatgagatatccaaaaagcaaaaaagaaaaacaaaacaaaacagagaaacctacaggaaaatccaaacagaaaaggcaaagaaagaacccgaactgggccaggcaatgtttccaacggcctcgctcttcctgaacaagaaggccagtcagcccatgggctgctcccagtactcgggccccgctgtggcagcacgccatgtaatagttttcgcgggaatccaacgccgaaatcgcccgcagcgggaacccgacgtcggtctggtgcgttctggcgccttccagaactctccacaggctcccgcagccgtccgatcagatcagcacgaagcacgaacattggcgcgcggcgatattttctttcctcgcccgacgacggccgcactgcatttcattttgaatttcaaaattcggaaacggaaaagctttctcgcatcccgaggcgaggcggttacgggcgccagaggggccaccccacccacccacccccgccctcacgtgccccgcgcggccgcatccgggccgtccgcgcggacagctggccgcgcccagcccgaaccgacgcccaggatcgagcgagggcggcgcgcccggggcttggcttagcgtccacgccacctccggctatataagccgccccacacccgctccccctccggcattccattccgccaccgcaccaccaccaccaccaaaccctagcgagcgagcgagggagagagagaccgccccgccgcgacg

SEQ ID NO: 7 - DNA, 4335 bp, Triticum aestivum
  exon (1528)..(1855)
  exon (2925)..(3008)
  exon (3133)..(3380)
agacttaaaccatttagttacaaatatcgatgcacaccttcggtggggcgttgtgaaaaagcatgttttttgggtcgacaagccccttttgcaacgtatcctcttctaatcctattcagatcattaacatcataagctgcaattgacatgctcttctgaggatcaggttcatgcaattaaacatcataaactgcatctttgatgtcatccttttcctatattttttccagattattggcttgcttcgttttcaatatcaggttctatgattcgacttctgttgttgccagtaataatttgtagttgctgcggaatatgaactcaaggagagctgatggtgctatgaagttgatttgatgggaggttgttctacacctgcacttgctgctcgacttaaatacatgccttggatttcttcccagctctagtacataatatttttcaaattaatgttccacgacataaaatttaaatccacaaacatatttttagtacatgaacaattttctaatatagggcaaacatttttcatatacaaaccgatcattttaatatatggtgaaaatcagtgtaatatatgctgaaatgttttcaaatacatattgaacatatttataataaatggtgaacattttttttaataattgatgaccatttttaaaatgcatattgaacattttataatatacactgtacagttttataataatcgacgaacatcttttggagttctgaacatttttttcaaaaacacaagccattttccaggaagaatacaaatgcaaaagaaatgagatatccaaaaagcaaaaaagaaaaacaaaacaaaacagagaaacctacaggaaaatccaaacagaaaaggcaaagaaagaacccgaactgggccaggcaatgtttccaacggcctcgctcttcctgaacaagaaggccagtcagcccatgggctgctcccagtactcgggccccgctgtggcagcacgccatgtaatagttttcgcgggaatccaacgccgaaatcgcccgcagcgggaacccgacgtcggtctggtgcgttctggcgccttccagaactctccacaggctcccgcagccgtccgatcagatcagcacgaagcacgaacattggcgcgcggcgatattttctttcctcgcccgacgacggccgcactgcatttcattttgaatttcaaaattcggaaacggaaaagctttctcgcatcccgaggcgaggcggttacgggcgccagaggggccaccccacccacccacccccgccctcacgtgccccgcgcggccgcatccgggccgtccgcgcggacagctggccgcgcccagcccgaaccgacgcccaggatcgagcgagggcggcgcgcccggggcttggcttagcgtccacgccacctccggctatataagccgccccacacccgctccccctccggcattccattccgccaccgcaccaccaccaccaccaaaccctagcgagcgagcgagggagagagagaccgccccgccgcgacgatggagagatcccgcgggctgctgctggtggcggggctgctggcggcgctgctgccggcggcggcggcgcagccgggggcgccgtgcgagcccgcgctgctggcgacgcaggtggcgctcttctgcgcgcccgacatgccgacggcccagtgctgcgagcccgtcgtcgccgccgtcgacctcggcggcggggtgccctgcctctgccgcgtcgccgccgagccgcagctcgtcatggcgggcctcaacgccacccacctcctcacgctctacagctcctgcggcggcctccgccccggcggcgcccacctcgccgccgcctgcgaaggtacgttgtccgcctcctcccctccctccctccctccctctctctctacgtgctcgctttcctgcttacctagtagtacgtagtttcccatgccttcttgactcgctagaagtgctccggtttgggtctgttaatttcctcgctgtactaccggatctgtcgtcggcacggcgcgcggcgtcgggtcctcgccttctcccgtggcgaccgacctgcgcagcgcgcgcgcggcctagctagcttcataccgctgtacctcgacatacacggagcgatctatggtctactctgagtatttcctcatcgtagaacgcatgcgccgctcgcgattgtttcgtcgattctagatccgtgcttgttcccgcgagttagtatgcatctgcgtgcatatgccgtacgcacgcagatgcagagtctgttgctcgagttatctactgtcgttcgctcgaccatatttgcctgttaatttcctgttcatcgtgcatgcagtagtagtagccatgtccacgccttcttgttttgaggcgatcatcgtcgagatccatggctttgctttctgcactatcttctgccttgttttgttctccgcagtacgtacgtcttgcttggtcaaaactgaaaaacgctttgctgtttgtttgatcggcaagagctggccgtgcttttggcaccgcagtgcgtcgcctctgccgcttttgcgaaacatttccatgttgatcctctggcggaactactttttcgcgtgcggtttgcgtggccttcctctctcgtgaaaagaggtcgggtcaaaccaaatggatcgcctcttggcagagcagcggcagcagatagctggccgtctcgcagctttggcagaaccggtctgtggccatctgtcgccgcctgccaccgtttccctgatgtttgtttctctctcgcctgccactgtttcttttcttgttgcgcacgtacgtcgtcacctcctcctacttttttgccagttttgtttacttttgatgaaatatacggatgaatcggctggtgattaactttggctgctgctgttaattactgtggattttggatgcaggacccgctcccccggccgccgtcgtcagcagccccccgcccccgcctccaccgtccgccgcacctcgccgcaagcagccagcgcgtaagaacctctccctctccctctctctctccctctcgcctgcatctcgctatgtttatccatgtccatatgttgatcagccttgtttagttactaacatgtgcaccggatcgggttctcgcagacgacgcaccaccgccgccaccgccgtcgagcgagaagccgtcgtccccgccgccgtcccaggaccacgacggcgccgccccccgcgccaaggccgcgcccgcccaggcggccacctccacgctcgcgcccgccgccgccgccaccgccccgccgccccaggcgccgcactccgccgcgcccacggcgccgtccaaggcggccttcttcttcgtcgccacggccatgctcggcctctacatcatcctctgagtcgcgcgccgaccccgcgagagaccgtggtccgtccagtcgcagtagagtagagcgctcgtcgtctcgttccgtttcgtgcctgtcgccgttcgaggttcgtttctgcgtgcagtccggtcgaagaagccggtgggttttgagtactagtggtagtagtagcagcagctatcgtttctgtccgctcgtacgtgtttgcgtggtcgcggagaacaattaattgggtgtttgcgagtcctctggttaagatgaaccactgatgctatgtgatcgatcgatcggtatgatctgaatggaaatggatcaagttttgcgttctgctgatgatgtgatccatttggatctgtgtggggcaacagtttcgcttgcttttgctctgcgatgaacgaatgcttcttgcatgcatcttgtctttgcttaatttgaactgtagaacggatgcagtactgatttctgcttatgatgtgacgattcgtcgtacgcatatcatctcttcaaatttgtgtagcagctgtttgtagcttccattctgctatggacgaatgcctgtttttcacggagaaccgcgcgcggggaccgatgcggctttgtgttgccatgttgttttccacgccaggacaaaatagatggtgcggttttgatccccaatcccaccatcaccatgttccggagagccacatggaactcacgtcaagcggtcactttttgcagaatcactcttaccattttacccttttgttgaaacctctctcctcatccccaaaagttgatgcaacagtgctatgcgcgcccacccatgctttttcatatgattgtaaaatttggatcgattttatcttttgaaccctaagtccggtttacaatctgtttgcatgtttatgttccttgcggcgaggaccattaaacaagactactattggatatatttcgacaggctttgaaatccgaattc

SEQ ID NO: 8 - DNA, 1527 bp, Artificial Sequence
  synthesized
aagcttaaaccatttagttacaaatatcgatgcacaccttcggtggggcgttgtgaaaaagcatgttttttgggtcgacaagccccttttgcaacgtatcctcttctaatcctattcagatcattaacatcataagctgcaattgacatgctcttctgaggatcaggttcatgcaattaaacatcataaactgcatctttgatgtcatccttttcctatattttttccagattattggcttgcttcgttttcaatatcaggttctatgattcgacttctgttgttgccagtaataatttgtagttgctgcggaatatgaactcaaggagagctgatggtgctatgaagttgatttgatgggaggttgttctacacctgcacttgctgctcgacttaaatacatgccttggatttcttcccagctctagtacataatatttttcaaattaatgttccacgacataaaatttaaatccacaaacatatttttagtacatgaacaattttctaatatagggcaaacatttttcatatacaaaccgatcattttaatatatggtgaaaatcagtgtaatatatgctgaaatgttttcaaatacatattgaacatatttataataaatggtgaacattttttttaataattgatgaccatttttaaaatgcatattgaacattttataatatacactgtacagttttataataatcgacgaacatcttttggagttctgaacatttttttcaaaaacacaagccattttccaggaagaatacaaatgcaaaagaaatgagatatccaaaaagcaaaaaagaaaaacaaaacaaaacagagaaacctacaggaaaatccaaacagaaaaggcaaagaaagaacccgaactgggccaggcaatgtttccaacggcctcgctcttcctgaacaagaaggccagtcagcccatgggctgctcccagtactcgggccccgctgtggcagcacgccatgtaatagttttcgcgggaatccaacgccgaaatcgcccgcagcgggaacccgacgtcggtctggtgcgttctggcgccttccagaactctccacaggctcccgcagccgtccgatcagatcagcacgaagcacgaacattggcgcgcggcgatattttctttcctcgcccgacgacggccgcactgcatttcattttgaatttcaaaattcggaaacggaatagctttctcgcatcccgaggcgaggcggttacgggcgccagaggggccaccccacccacccacccccgccctcacgtgccccgcgcggccgaatccgggccgtccgcgcggacagctggccgcgcccagcccgaaccgacgcccaggatcgagcgagggcggcgcgcccggggcttggcttagcgtccacgccacctccggctatataagccgccccacacccgctccccctccggcattccattccgccaccgcaccaccaccaccaccaaaccctagcgagcgagcgagggagagagagaccgccccgccgcgacg

SEQ ID NO: 9 - DNA, 4335 bp, Artificial Sequence
  synthesized
aagcttaaaccatttagttacaaatatcgatgcacaccttcggtggggcgttgtgaaaaagcatgttttttgggtcgacaagccccttttgcaacgtatcctcttctaatcctattcagatcattaacatcataagctgcaattgacatgctcttctgaggatcaggttcatgcaattaaacatcataaactgcatctttgatgtcatccttttcctatattttttccagattattggcttgcttcgttttcaatatcaggttctatgattcgacttctgttgttgccagtaataatttgtagttgctgcggaatatgaactcaaggagagctgatggtgctatgaagttgatttgatgggaggttgttctacacctgcacttgctgctcgacttaaatacatgccttggatttcttcccagctctagtacataatatttttcaaattaatgttccacgacataaaatttaaatccacaaacatatttttagtacatgaacaattttctaatatagggcaaacatttttcatatacaaaccgatcattttaatatatggtgaaaatcagtgtaatatatgctgaaatgttttcaaatacatattgaacatatttataataaatggtgaacattttttttaataattgatgaccatttttaaaatgcatattgaacattttataatatacactgtacagttttataataatcgacgaacatcttttggagttctgaacatttttttcaaaaacacaagccattttccaggaagaatacaaatgcaaaagaaatgagatatccaaaaagcaaaaaagaaaaacaaaacaaaacagagaaacctacaggaaaatccaaacagaaaaggcaaagaaagaacccgaactgggccaggcaatgtttccaacggcctcgctcttcctgaacaagaaggccagtcagcccatgggctgctcccagtactcgggccccgctgtggcagcacgccatgtaatagttttcgcgggaatccaacgccgaaatcgcccgcagcgggaacccgacgtcggtctggtgcgttctggcgccttccagaactctccacaggctcccgcagccgtccgatcagatcagcacgaagcacgaacattggcgcgcggcgatattttctttcctcgcccgacgacggccgcactgcatttcattttgaatttcaaaattcggaaacggaatagctttctcgcatcccgaggcgaggcggttacgggcgccagaggggccaccccacccacccacccccgccctcacgtgccccgcgcggccgaatccgggccgtccgcgcggacagctggccgcgcccagcccgaaccgacgcccaggatcgagcgagggcggcgcgcccggggcttggcttagcgtccacgccacctccggctatataagccgccccacacccgctccccctccggcattccattccgccaccgcaccaccaccaccaccaaaccctagcgagcgagcgagggagagagagaccgccccgccgcgacgatggagagatcccgcgggctgctgctggtggcggggctgctggcggcgctgctgccggcggcggcggcgcagccgggggcgccgtgcgagcccgcgctgctggcgacgcaggtggcgctcttctgcgcgcccgacatgccgacggcccagtgctgcgagcccgtcgtcgccgccgtcgacctcggcggcggggtgccctgcctctgccgcgtcgccgccgagccgcagctcgtcatggcgggcctcaacgccacccacctcctcacgctctacagctcctgcggcggcctccgccccggcggcgcccacctcgccgccgcctgcgaaggtacgttgtccgcctcctcccctccctccctccctccctctctctctacgtgctcgctttcctgcttacctagtagtacgtagtttcccatgccttcttgactcgctagaagtgctccggtttgggtctgttaatttcctcgctgtactaccggatctgtcgtcggcacggcgcgcggcgtcgggtcctcgccttctcccgtggcgaccgacctgcgcagcgcgcgcgcggcctagctagcttcataccgctgtacctcgacatacacggagcgatctatggtctactctgagtatttcctcatcgtagaacgcatgcgccgctcgcgattgtttcgtcgattctagatccgtgcttgttcccgcgagttagtatgcatctgcgtgcatatgccgtacgcacgcagatgcagagtctgttgctcgagttatctactgtcgttcgctcgaccatatttgcctgttaatttcctgttcatcgtgcatgcagtagtagtagccatgtccacgccttcttgttttgaggcgatcatcgtcgagatccatggctttgctttctgcactatcttctgccttgttttgttctccgcagtacgtacgtcttgcttggtcaaaactgaaaaacgctttgctgtttgtttgatcggcaagagctggccgtgcttttggcaccgcagtgcgtcgcctctgccgcttttgcgaaacatttccatgttgatcctctggcggaactactttttcgcgtgcggtttgcgtggccttcctctctcgtgaaaagaggtcgggtcaaaccaaatggatcgcctcttggcagagcagcggcagcagatagctggccgtctcgcagctttggcagaaccggtctgtggccatctgtcgccgcctgccaccgtttccctgatgtttgtttctctctcgcctgccactgtttcttttcttgttgcgcacgtacgtcgtcacctcctcctacttttttgccagttttgtttacttttgatgaaatatacggatgaatcggctggtgattaactttggctgctgctgttaattactgtggattttggatgcaggacccgctcccccggccgccgtcgtcagcagccccccgcccccgcctccaccgtccgccgcacctcgccgcaagcagccagcgcgtaagaacctctccctctccctctctctctccctctcgcctgcatctcgctatgtttatccatgtccatatgttgatcagccttgtttagttactaacatgtgcaccggatcgggttctcgcagacgacgcaccaccgccgccaccgccgtcgagcgagaagccgtcgtccccgccgccgtcccaggaccacgacggcgccgccccccgcgccaaggccgcgcccgcccaggcggccacctccacgctcgcgcccgccgccgccgccaccgccccgccgccccaggcgccgcactccgccgcgcccacggcgccgtccaaggcggccttcttcttcgtcgccacggccatgctcggcctctacatcatcctctgagtcgcgcgccgaccccgcgagagaccgtggtccgtccagtcgcagtagagtagagcgctcgtcgtctcgttccgtttcgtgcctgtcgccgttcgaggttcgtttctgcgtgcagtccggtcgaagaagccggtgggttttgagtactagtggtagtagtagcagcagctatcgtttctgtccgctcgtacgtgtttgcgtggtcgcggagaacaattaattgggtgtttgcgagtcctctggttaagatgaaccactgatgctatgtgatcgatcgatcggtatgatctgaatggaaatggatcaagttttgcgttctgctgatgatgtgatccatttggatctgtgtggggcaacagtttcgcttgcttttgctctgcgatgaacgaatgcttcttgcatgcatcttgtctttgcttaatttgaactgtagaacggatgcagtactgatttctgcttatgatgtgacgattcgtcgtacgcatatcatctcttcaaatttgtgtagcagctgtttgtagcttccattctgctatggacgaatgcctgtttttcacggagaaccgcgcgcggggaccgatgcggctttgtgttgccatgttgttttccacgccaggacaaaatagatggtgcggttttgatccccaatcccaccatcaccatgttccggagagccacatggaactcacgtcaagcggtcactttttgcagaatcactcttaccattttacccttttgttgaaacctctctcctcatccccaaaagttgatgcaacagtgctatgcgcgcccacccatgctttttcatatgattgtaaaatttggatcgattttatcttttgaaccctaagtccggtttacaatctgtttgcatgtttatgttccttgcggcgaggaccattaaacaagactactattggatatatttcgacaggctttgaaatccgaattc

SEQ ID NO: 10 - DNA, 241 bp, Hordeum vulgare
  variation (121)..(121): a or c
ttttacagcagcaacaacaacaacaaaacccaagtcaccagtaagagcttacacgcagcctgagggcgggcacgacacaaacgggtataaggttgacacgtacatccaacacagggcaaamaagttccgtttcaaggggtcgcgagcccggagttccaccgctggaatcggtcaatccggttctgcacacacacagccgttacactgcctacaaacaagtttaagggatacatacacactg

SEQ ID NO: 11 - DNA, 274 bp, Triticum aestivum
  variation (34)..(34): c (Chris) or t (Gladius)
  variation (54)..(54): g (Chris) or t (Gladius)
  variation (83)..(83): t (Chris) or c (Gladius)
  variation (130)..(130): g (Chris) or a (Gladius)
  variation (165)..(165): a (Chris) or gap (Gladius)
  variation (174)..(174): a (Chris) or t (Gladius at 173)
  variation (186)..(186): t (Chris) or g (Gladius at 185)
  variation (253)..(253): t (Chris) or c (Gladius at 252)
atgatggatggacggatgatgctctgtggtgccytgtatttatatttgttgagktctttgatacaggatgatatgtctccaaygtatctataattttttgttgttccatgttgttatattatcattttgratgttttacaatcattttataatcattctatatcattttttgtwactaacctattkacatagtgccaagtgctagttgttgttttctgcttgttttttacatcgcaggaaatcaataccaaayggagtccaaacgcagcaaaac

SEQ ID NO: 12 - DNA, 273 bp, Triticum aestivum
atgatggatggacggatgatgctctgtggtgccttgtatttatatttgttgagttctttgatacaggatgatatgtctccaacgtatctataattttttgttgttccatgttgttatattatcattttgaatgttttacaatcattttataatcattctatatcttttttgttactaacctattgacatagtgccaagtgctagttgttgttttctgcttgttttttacatcgcaggaaatcaataccaaacggagtccaaacgcagcaaaac

SEQ ID NO: 13 - DNA, 274 bp, Triticum aestivum
atgatggatggacggatgatgctctgtggtgccctgtatttatatttgttgaggtctttgatacaggatgatatgtctccaatgtatctataattttttgttgttccatgttgttatattatcattttggatgttttacaatcattttataatcattctatatcattttttgtaactaacctatttacatagtgccaagtgctagttgttgttttctgcttgttttttacatcgcaggaaatcaataccaaatggagtccaaacgcagcaaaac

SEQ ID NO: 14 - DNA, 415 bp, Aegilops speltoides
accaggcctcccgaccccaccgtgagcatgcgcttcgcgtgcacggcggcaccactccgctacggcctcggcccttcttcttccttctccgacaacgccgcctcctcgtgttgttcttcttcgtctcggattctatctacaaggagctagctagctagcgcgattcactgatctctagctggggaggggtacaaccgtacaagcatggagcccggagctttagcgacgtgcggggcggtggccttctcctgggagcaggagccgggggtgtccaaggagagcccggcggccgaggcgaggaagccctccggtggaaggacgccggacagcaccaggaaggtggaggtgcagacggacaggctgctcgtgccccctccaccgggagggcccggagcgccgtctctgtcgccggtga

SEQ ID NO: 15 - DNA, 281 bp, Triticum aestivum
  variation (224)..(224): t (Chris) or a (Gladius)
  variation (229)..(229): c (Chris) or a (Gladius)
  variation (253)..(253): a (Chris) or c (Gladius)
ttaatagtgttccgccctgcgtggcacagaccgtaacgaatgattgtacgaacgtttttcactaatcattacataggtgtggtttaagaaaaaatcaaccaccttaacgccgtaatcccctctacagaataaccacacaagtcatgaaaaggaactattaacaaaaatagatgataaaataaatctcaaatccaaattcataaagcacctctagtctataaacwcgacmaatctagctatgtttagtacttcmtccgttccaaaatacttgtcgtggtttt

SEQ ID NO: 16 - DNA, 281 bp, Triticum aestivum
ttaatagtgttccgccctgcgtggcacagaccgtaacgaatgattgtacgaacgtttttcactaatcattacataggtgtggtttaagaaaaaatcaaccaccttaacgccgtaatcccctctacagaataaccacacaagtcatgaaaaggaactattaacaaaaatagatgataaaataaatctcaaatccaaattcataaagcacctctagtctataaacacgacaaatctagctatgtttagtacttcctccgttccaaaatacttgtcgtggtttt

SEQ ID NO: 17 - DNA, 281 bp, Triticum aestivum
ttaatagtgttccgccctgcgtggcacagaccgtaacgaatgattgtacgaacgtttttcactaatcattacataggtgtggtttaagaaaaaatcaaccaccttaacgccgtaatcccctctacagaataaccacacaagtcatgaaaaggaactattaacaaaaatagatgataaaataaatctcaaatccaaattcataaagcacctctagtctataaactcgaccaatctagctatgtttagtacttcatccgttccaaaatacttgtcgtggtttt

SEQ ID NO: 18 - DNA, 199 bp, Triticum aestivum
  variation (101)..(101): t (Gladius) or c (Chris)
atgctcatggtgcacgcgacgagaagtggccagagacaatccttgaccatgatcgaataatatggctcggggatttgaattaccggatagcgctttcctaycgctctgtgaaggctttggttgagatgcacaattggaaacaattgttggaaaaagatcagcttcgtatagagcaaaggtttggtcgggtattcgcggg

SEQ ID NO: 19 - DNA, 199 bp, Triticum aestivum
atgctcatggtgcacgcgacgagaagtggccagagacaatccttgaccatgatcgaataatatggctcggggatttgaattaccggatagcgctttcctatcgctctgtgaaggctttggttgagatgcacaattggaaacaattgttggaaaaagatcagcttcgtatagagcaaaggtttggtcgggtattcgcggg

SEQ ID NO: 20 - DNA, 199 bp, Triticum aestivum
atgctcatggtgcacgcgacgagaagtggccagagacaatccttgaccatgatcgaataatatggctcggggatttgaattaccggatagcgctttcctaccgctctgtgaaggctttggttgagatgcacaattggaaacaattgttggaaaaagatcagcttcgtatagagcaaaggtttggtcgggtattcgcggg

SEQ ID NO: 21 - DNA, 198 bp, Triticum aestivum
  variation (101)..(101): a (Gladius) or g (Chris)
  variation (165)..(165): c (Gladius) or t (Chris)
tatatgaattaggctttgcggaccggaagtacaacgccaacttgcttggtgttcctgcactgctgcttgagaccttgatgtgcaaagttatgaacatatcrgcgtaactagggaaagtgaatatgtataatactagcaaacaagttagattaggctaaatcgcgytattttccggtgagctgggatttcctggccagt

SEQ ID NO: 22 - DNA, 198 bp, Triticum aestivum
tatatgaattaggctttgcggaccggaagtacaacgccaacttgcttggtgttcctgcactgctgcttgagaccttgatgtgcaaagttatgaacatatcagcgtaactagggaaagtgaatatgtataatactagcaaacaagttagattaggctaaatcgcgctattttccggtgagctgggatttcctggccagt

SEQ ID NO: 23 - DNA, 198 bp, Triticum aestivum
tatatgaattaggctttgcggaccggaagtacaacgccaacttgcttggtgttcctgcactgctgcttgagaccttgatgtgcaaagttatgaacatatcggcgtaactagggaaagtgaatatgtataatactagcaaacaagttagattaggctaaatcgcgttattttccggtgagctgggatttcctggccagt

SEQ ID NO: 24 - DNA, 58 bp, Triticum aestivum
  variation (22)..(22): t (Chris) or c (Gladius)
atgtggaccttggcaagatttyatatgcattttgagagaaatagaagtaatgtgattg

SEQ ID NO: 25 - DNA, 56 bp, Triticum aestivum
  variation (27)..(27): g (Chris) or a (Gladius)
ggttttgggtttactttgagtcatagragaagccatactataaagagggggttgct

SEQ ID NO: 26 - DNA, 53 bp, Triticum aestivum
  variation (31)..(31): t (Chris) or g (Gladius)
acttgattgtactttttggttagcaacaatkgcaatgacttgacaagggaaag

SEQ ID NO: 27 - DNA, 50 bp, Triticum aestivum
  variation (30)..(30): g (Chris) or c (Gladius)
ctcgccttggctatagggtcctctgtgagsaaggaaaaggtcgaggaggc

SEQ ID NO: 28 - DNA, 59 bp, Triticum aestivum
  variation (38)..(38): a (Chris) or g (Gladius)
caacgctatcccttaaaacggatacactatccatccgrgaagcatgttcggatgtgttg

SEQ ID NO: 29 - DNA, 39 bp, Triticum aestivum
  variation (20)..(20): a (Chris) or G (Gladius)
ctcgccgccgcctgcgaagrtacgttgtccgcctcctcc

SEQ ID NO: 30 - DNA, 1618 bp, Zea mays
  CDS (108)..(1430)
ggcacgagccggcgagcccactcggcagtcggcacaaccacacacacctccacccactctctgagataagtgaagcatctcgcgcactgtcgcagtcgcagacggagatgatgaagcactcgagcagcttgtgcttgctcttcctcttggcgctctgcaccaccctgctggcctgcggcctggtccaggcacaagtcctcttccaggggtttaactgggagtcgtgcaagcagcagggaggctggtacaacaggctcaaggcccaggtcgacgacatcgccaaggccggcgtcacgcacgtctggctgcctccaccctcgcactccgtctcgccacaaggctacatgccaggccgcctatacgacctggacgcgtccaagtacggcacggcggcggagctcaagtccctgatagcggcgttccacggcaggggcgtgcagtgcgtggcggacatcgtcatcaaccaccggtgcgcggaaaagaaggacgcgcgcggcgtgtactgcatcttcgagggcgggactcccgacgaccgcctggactggggccccgggatgatctgcagcgacgacacgcagtactcggacgggacggggcaccgcgacacgggcgaggggttcgcggcggcgcccgacatcgaccacctcaacccgcgcgtgcagcgggagctctccgcctggctcaactggctcaggtccgacgccgtggggttcgacggctggcgcctcgacttcgccaagggctactcgccggccgtcgccagaatgtacgtggagagcacggggccgccgagcttcgtcgtcgcggagatatggaactcgctgagctacagcggggacggcaagccggcgcccaaccaggaccagtgccggcaggagctgctggactggacgcgggccgtcggcgggcccgccatggcgttcgacttccccaccaagggcctgctgcaggcgggcgtgcagggggagctgtggcggctgcgcgacagctccggcaacgcggccggcctgatcgggtgggcgcccgagaaggccgtcaccttcgtcgacaaccatgacaccgggtcgacgcagaagctctggccgttcccatccgacaaggtcatgcagggctacgcctacatcctcacccatccaggagtcccctgcattttctacgaccacatgttcgactggaacctgaagcaggagatatccacgctgtctgccatcagggcgcggaacggcatccgcgccgggagcaagctgcggatcctcgtggcggacgcggacgcgtacgtggccgtcgtcgacgagaaggtcatggtgaagatcgggacaaggtacggcgtgagcagcgtggtcccgtcggatttccacccggcggcgcacggcaaggactactgcgtctgggagaaagcgagcctccgcgtcccggcggggcgccacctctagcagctcagattgctcagtcttgtgctgcattgcaaacacagcagcacgacactgcataacgtcttttccttaatttcctgaattttaccttttcctagttcaatttcatatatgtatttctacatgtacacactatcacaatcagataaataaacaagcttggtcaaaaaaaaaaaaaaaaaaaa

SEQ ID NO: 31 - protein, 441 aa, Zea mays
MMKHSSSLCLLFLLALCTTLLACGLVQAQVLFQGFNWESCKQQGGWYNRLKAQVDDIAKAGVTHVWLPPPSHSVSPQGYMPGRLYDLDASKYGTAAELKSLIAAFHGRGVQCVADIVINHRCAEKKDARGVYCIFEGGTPDDRLDWGPGMICSDDTQYSDGTGHRDTGEGFAAAPDIDHLNPRVQRELSAWLNWLRSDAVGFDGWRLDFAKGYSPAVARMYVESTGPPSFVVAEIWNSLSYSGDGKPAPNQDQCRQELLDWTRAVGGPAMAFDFPTKGLLQAGVQGELWRLRDSSGNAAGLIGWAPEKAVTFVDNHDTGSTQKLWPFPSDKVMQGYAYILTHPGVPCIFYDHMFDWNLKQEISTLSAIRARNGIRAGSKLRILVADADAYVAVVDEKVMVKIGTRYGVSSVVPSDFHPAAHGKDYCVWEKASLRVPAGRHL

SEQ ID NO: 32 - DNA, 55 bp, Triticum aestivum
  variation (30)..(30): c (Gladius) or a (Chris)
atcacattgcacaagttaatagtccggtamtgggtaattacctttggactttcca

SEQ ID NO: 33 - DNA, 61 bp, Triticum aestivum
  variation (27)..(27): a (Gladius) or t (Chris)
tgtttctgctgcttgctctgcttatawaatgataatgatatgtgcgaatggtctgttcatg

SEQ ID NO: 34 - DNA, 45 bp, Artificial Sequence
  Flanking marker amplicon
ggttttccctagtagtgtgaggrgaacgcctcatcccactcgctc

SEQ ID NO: 35 - DNA, 61 bp, Artificial Sequence
  Flanking marker 007-0011.1 amplicon
gtatatactagtaaatcaataaggtcgatrctaaagatagaaaaatacctgaagtggtgcc

SEQ ID NO: 36 - DNA, 44 bp, Artificial Sequence
  amplicon
ggcctaaaatttgagcccgaaggttgrgccgggcttgggcttga

SEQ ID NO: 37 - DNA, 79 bp, Artificial Sequence
  amplicon
tcattttgaatttcaaaattcggaaacggaawagctttctcgcatcccgaggcgaggcggttacgggcgccagaggggc

SEQ ID NO: 38 - DNA, 196 bp, Triticum aestivum
tgtcgccgttcgaggttcgtttctgcgtgcagtccggtcgaagaagccggtgggttttgagtactagtggtagtagtagcagcagctatcgtttctgtccgctcgtacgtgtttgcgtggtcgcggagaacaattaattgggtgtttgcgagtcctctggttaagatgaaccactgatgctatgtgatcgatcgat

SEQ ID NO: 39 - protein, 228 aa, Brachypodium distachyon
MERSHHLLLVLGLLAALLPAAAATFGTTQPEPGAPCEPTLLATQVSLFCAPDMPTAQCCEPVVASVDLGGGVPCLCRVAAEPQLVMAGLNATHLLTLYTSCGGLRPGGAHLAAACEGPAPPAAVVSAPPPSAAPRRKQPAHEAPPPPPSTEKPSPPPQQDNVTAHGKAIPTHAATSPLAPAASMIHMSPPPACNPCSGSAASSAEGPLLIAALLLVITAIIVGTLDDK

SEQ ID NO: 40 - protein, 228 aa, Oryza sativa
MERSHLAVLLGLLAFAAGVPAAAAATAVEGAQAATAEASCEPSILATQVSLFCAPDMPTAQCCEPVVASVDLGGGVPCLCRVAAEPQLIISGLNATHLLTLYAACGGLRPGGARLAAACEGPAPPASIVTAPPPPVAFRRKPPAREAPPPPPAAEKLSPPPQQHDDSDHNKRVGPLPRGSPPPYAQSVPVGPAAAPPPPRSGASSSLQAPLAATTTIVAITLIAAAQY

SEQ ID NO: 41 - DNA, 902 bp, Hordeum vulgare
cgcacatcaacataaactcatcagatgggaataatcggatctacgaaggacataaaactctttaatctcatgacaacgccagaagagcaagagtaaatatattctcataaaaaacaatgaacactagatgatgacgaagaacataagattcttcaaggagaaattgcggcagcggagatggcagccggaggcgagggggccaaaaactctgttgcggcggcagcggtagccttggtgaaacccacacgtttgcacaccatataagttgtttgcaagggttacatgggcctcgctctcgtgaaaaagaaggtcatacatgggtcttggtctcgtgcaaaacgaaaggtcagcagtccatgggccggaggaaaaaccgggcaacaacacgccatgtgtgttttcgcgggaacccaattccgaaatcactcaccggcacctcgtcccgatgccttccagaacgttctacgtgcttccacagggccagcccagccgtgggatcagatcaggatcagcacgaacattgaagctagcgcggcgatatttttcccagcctccgcctcgctcgacgactgcatttcatttcgaaaacaaaaaaaagagctttctccttctcatcccgagcgccagaggagcaccagaaaggccacccacccaccctcacgtaccgccctcgcacccgcgcggccacatctgggccgtccacttgggcagctggccgttccattcccgaactgacgggcaggatcgagcgagcggcgcgcccacggctcctccggctatataacccgccacccacaccactcccctccggcgttccaccagagccttcctccctccaccgcaccaccaccaccaccgcgccaaaaaccctagggagcgagcgagctcacctcgccccgccc

SEQ ID NO: 42 - DNA, 4504 bp, Oryza sativa
  exon (1001)..(1363)
  exon (3093)..(3164)
  exon (3253)..(3505)
gaacagtgcactggttgggataacaagaagttagaaattgggcatatatatagaagggtaagacacctctaatggatagggtggacaatccatcaaagatgactattttggcacctctgaggccgtgacaagttgcctatcttcgcacccttcacaagtgactccctacttgtgatgggtcgtgagatgtgagccggtgatctttctcagatgtaaatttcggcctctcacaagtgactccttatctgtgataggtcttgccctcacagcctcatctgtaacggcctctaattcaatccgttacagattaaatcattcatgacaagacactttgacccatcataggtgggttgttaatgttgaaccgaggtagcgtggtggtggcttctttgattgttgagcgggttgtgttcttcatcacttggtaggaagtaggaacccaagaaggttagaagcccacaactattatatcgtcggcctcattggtaaatgggctagaagcctagaggcaatctgattcaatagtgtcggaaatttgtggatgggccagagacgttgcgtcgtcttcgactcttcgagtgcctggcctacggatctgcacgaatcttagagcaagtagaaaatcgcatatcgtcgtgtagagcgcagcacaaattcgagttgcttttccctttttcgcagccaaatcttacctgctcacgtgccgtgctgcccggtgtgcagagcccacgcgccacggcgccagtgtactacaccgaatcggcaccatccatcgccacagctggccggtcccccctaagacggacgctccggatcaatccacgttggcatggcttccccgcatcgccttctccgcgcccccgcctatataatggcgctctcgcttctcttccccatttcgtcttccccttctctagagccttcctctcacagagcacacacaaaaccctagagtaggaagcgagcgagagagagagagagagagagagagaccacacccatggagcgctcccacctcgccgtcctgctcggcctcctcgccttcgccgccggggtcccggccgcagcggcggccaccgccgtggagggagcgcaggcggccacggcggaggcgtcgtgcgagccctccatcctcgccacccaggtctcgctcttctgcgcgcccgacatgcccaccgcgcagtgctgcgagccggtggtggcctccgtcgacctcggcggcggcgtaccctgcctctgccgcgtcgccgccgagccgcagctcatcatctccggcctcaacgccacccacctcctcacgctgtacgccgcctgcggaggcctccgccctggaggcgctcgcctcgccgccgcctgtgaaggtacgtacatgcataacctcctcctcctcctcctcctctctctctctctctctctctctctctctctctctctctctctctctctctctctctctctctctctctctctctctctctctctctctctctctctctctctctctctcggttggggttgctgccttgcgtttttggttggtttttcgtgggttgggcgagatccttcgagttgcttgtgttttgtggtatgctaggcttcgaacgagttgccggcgttgctgtgtcgaccaactctcgtatgcttatctttcagcacatgagttttggcctcgtttttactcggttgttgtatgctacttctgagatttgagttcatccactgctaaactgacatcatagatgaagaatagcagcggcgtttggtcgattttgattcctttctctggatgttcgagctgatcttgtggttattgctcgaagcctcgaaacgcttgcgcacatgcaagatccagcaacgtatagatctatagtggtgttgtgcttttattcggatttgtggttcagtgtttacgtgcgaagtcacgcgttcgatgtttccgcttgagctccatatctatagcacaaatcaatcatgtgcgttgcgcgagttcaagctcgagagaaaagaaaagcatcaaggccacggggggtttttgggccaggtcgtgattctcccttgaactccgaatataccgagtttattatcttttgagcggatttggtgttgaactggcaggactcaaaacccacccgtgggacgatcgttttcttttcctttcgctttgtgttctctgtctcctttccgtgaaatctctgcgtttcccttctggtgcttgttatagatgattctggatcgagccgtgtatgctcgtgcagtggtacgacttggcgatgaacgtgcttgcggagctagtcgcagttcatctttcttttttttttccctcgtttcttttctcggcgtttcattctctacacctcttctactcgccatgcatgttcatctctctccgtgttggtcctcatttggagccgattcgaaccgggcagcacagtgctttttttctgtttcgttttggaggtttccactttcgtgaaaaggaaagggtcaaatcgaatcgccccctgaaccatcctttgcagagcttttttggacgtttccgcctttcgtcagagaccatctgcactgcgcgtttctccccaactcgatcgattttgcagcttttaatcactttttagaaaaagtttttaatcactcgtcatcgatgtgatctcttgctctaattgcatcttctccgtaggattagcacttccatgcttcttgttttgtctgttcaattagccaagaaacgagtcagtataccttcaagatgcatgcagatttaaaatcggcactgctctttatcttgttcttgtttttgcaagttttggttggttcaaaacttatctcttctgcagcattgcctgctgtgtacagaaagttggcaggggcatcgtgcagcttttttgcctgctgtgtgtaacgttttctttccgtacgttgcgttccgtttcacgtcgcttacctctgtttcttggggcgcaagttatggcagtacagccgttgtttccacgttggaaggacggttttgccccttcgcttccagaagcttccagagatttttcgagtttttctaatgtgtttgttattgctgtaactcgttctaacgtgcaggtcccgccccaccggcctccatcgtcactgccccgccgcccccggttgcttttcgccgcaagccgccggcacgtaaggctgattgattccccttcatccactgattgttaatgcgcgtgtaatctttgtgattactaacttgctgctggatgctttgcaggcgaggcacctcccccaccgccggcggccgagaagctctccccgccgcctcagcagcacgacgactccgaccacaacaagcgcgtcggcccactcccgagaggctctcctcccccgtatgcccagtccgtcccggtcggccccgccgccgctcccccgccaccacgctccggcgcctcctcgtcgctccaggcgcccctcgccgccaccaccaccatcgttgccatcaccctcatcgccgccgcccagtactgaggacacgccgccgccggcgcccgctccccagagccatgattcgttcgcagtatttttcatcctgttcttttgcttctctctctggctacccatgtatatgagtttggaagacgatgatttgatctagtagcgcgttaccaagtttgcctagattcgagtagtagctgtggtactatgctgatgtctctttgatcgcgtcgtctctagagcgtccgccgtttttgatcgatcactagcatggccgatgtgagtccagcatgaaaagtggtcgaggagaacattgttgctaagttttttttttgctttctatctccagtagctgaacaagtatgtcaactgaatgctgcaatgaagtgaatggatgcagtcttaaatttagcctttctgttgccaacttcttcctctgttctgtacggttcagatgctgcttgttctgtttatgcgatggtgttgcattgttgtgatgtgtgaagtgcgcccaattctgggtgaactctgcagtattggcaagctctgatcgatacataaagaactgaaatgtgccggcttctccgcctcccgttgcatgctcttgtgcgcgagctgcacagcgcaaccgcgccctcctctgcacatccatcgacacaaagtctcaagttgttgcgcgtgtgctctaccaggcaccgtggctcctgcgggcgtgcacgggtcacattcacatcgcacccaagttgcggacgtttcagctgagcacctaccatccgcaatgtttgcccacagcttgctcgatgaaatgactggttcatgtcaaaaggtaaaaactgacattctcacgcggtaaattcccctaagcttcatagaccaccgcactgtcatccactcgacctgccacgacacccgccaccgcagaacgcgacaccctgtgcccacggccacctaccctggcacgcaccgagccgaagccggataagcacccgagttgatccccatgagacgtggcgactcggctgccctctgccac

SEQ ID NO: 43 - DNA, 684 bp, Oryza sativa
atggagcgctcccacctcgccgtcctgctcggcctcctcgccttcgccgccggggtcccggccgcagcggcggccaccgccgtggagggagcgcaggcggccacggcggaggcgtcgtgcgagccctccatcctcgccacccaggtctcgctcttctgcgcgcccgacatgcccaccgcgcagtgctgcgagccggtggtggcctccgtcgacctcggcggcggcgtaccctgcctctgccgcgtcgccgccgagccgcagctcatcatctccggcctcaacgccacccacctcctcacgctgtacgccgcctgcggaggcctccgccctggaggcgctcgcctcgccgccgcctgtgaaggtcccgccccaccggcctccatcgtcactgccccgccgcccccggttgcttttcgccgcaagccgccggcacgcgaggcacctcccccaccgccggcggccgagaagctctccccgccgcctcagcagcacgacgactccgaccacaacaagcgcgtcggcccactcccgagaggctctcctcccccgtatgcccagtccgtcccggtcggccccgccgccgctcccccgccaccacgctccggcgcctcctcgtcgctccaggcgcccctcgccgccaccaccaccatcgttgccatcaccctcatcgccgccgcccagtac

SEQ ID NO: 44 - DNA, 5291 bp, Brachypodium distachyon
  exon (2069)..(2419)
  exon (3818)..(3886)
  exon (4025)..(4288)
cccttaaaagggggtaatgatggctcatattgaggaattgacatgcaccccttaaaggaggtaatgatggctcatattgatttgaggaaactccttccataaggacatctccaacaagacacagtcagcggtactataaagcacggcacctggatcagttctcgtcgagggtgcagacgacgattgcagtgaatatgatgactatcgcggcgacgaggagggggggcagtggggacggctgaggtgcatcctctgccaaattaaagcacgcgcgcgtgccacgcgagtcagatcaaggacacgcaaaacagataacatattaacaggaagcaacgcatagatttttagaatcgagtaaaagaatagcagcagcattttttttagcgaaatagtagcagcaattagatcaagcgaaatgtaaaggttgttcacataccaacaagggcggcggtgtggggcgggacattgacctccggggcctcctccagggcctgcggcgcctgctgggcctcgacaaatgcagtcaggctgcaagatatgagggtaaaaaaacagatgtacagtccggtcaagaaaaacaacaaacatgcagactacttagatctgccaagactaaattacctaacgattccaagtccagtgatggttgcatcgcgatgaatttcagccatgctgcgtgcccgcctggttaccggacgcgcgggaaggggagcaagcccaatcagagcgggtgcagccgggcggcgtgtgttattgcgataatactcgacggtatgcttccaccgcaggtacagtctcaggaaggcatccgattgacccaccagatcatctatcaccaaggtagccattctgccacccatctaaacacaaactgagagtaagaaagcagtttgaccgcgattgtttatcacaaaaggcaacacaaaaaaactgctagcttcgtgtcagaaaatcaacatgcatggtgcgcgacagtacaacagaaacatggggagacatagcagaaacgtccaaaccaaaaatccaaaaaaagaaggagatgcactgcgtaagaaaacagcacgggaagcgctcttcaccgtgtgagactgcacaagtccaagagacgacaatagcagaaaagaactgcagaaaggagagctgctttcgggggtcaaagtactagcacggcttcgatcaatcggtcgattaaatccctcgtgccaccgagatcctcacagtgctcgaggggacactctaagtcggctttgtcacatccaacccaaacaacacgctcttgtctaaggtgctcaacaaaggtgatgtgttcgcacgcaggcacagtggaacaacaaactagcgtcgatcgaccacgtccctcccccagaaaagtgctcccaacatgatcgcatcgaagtaatcgtagagatagatcttacagaataaaaaataaacccaaaccaaaggaggagttctgcactactagatccgaaccaaagccaggaaatagcaaactaaacacaaaagatatcgatgaaatcatacatcgtccaaacgtttcggattacaccttctggtcgcaactctcgtgctcaccgcgcagacagatcttctgtacgtaccttggctccagcccgaggagagcgagcactccaggaaacggcggtctcgagcgagcagtctaggaaatggcggtcgcgatggaaaagccttcaagagatatcgggtgatgccccctatttctagagctctggcctttacagttcaccacttcaccctgcgccatcccgattcccagtacctatgacgagcgacgaccctcacgtgcctggccagcatcacgggagagaatcttgctcagcatctcaaccgcccaaacagacagctgtccggtcccacccaaatggacgcacaggatcgatcgggccgccggtggcctgtccttggctaacccttcacgcctcttcgtcccctccgcctatataatcccaccccgctccgcttcttcccccaccgcgctctcttcctctggactcacaccaactcgcctagccctagcggtaggaagcgaaagcgagagatcccacccatggagagatcccaccacctcctcctcgtgctcggcctcctcgccgcgctgctcccggcggccgcggctaccttcgggacgacgcagccggagcctggggccccatgcgagcccaccctcctcgccacccaggtctcgctcttctgcgcgccggacatgccgaccgcgcagtgctgcgagcctgtggtggcctccgtcgacctcgggggtggcgtcccctgcctctgccgtgtcgccgccgagccgcagctcgtcatggccggcctcaacgccacccacctcctcacgctctacacctcctgcggtggactccgccccggaggcgcccacctcgccgccgcctgtgaaggtacgcgacgcctgcgtctctctctctctctgcgtctctctctgcgtctctcccatgacgagcaactcgcgatacgccttactgccttattttttttgaagatatgtgtctgcttggtccactgtatttgggttcttctttcgagaagttcatccgtaggcatctataatccgacgagttcggatgagatcaaacagtgacacgcgcgacaccaacgttttcaacgatctcttgctgtttggtttgatatttcctgcttcccatgatctattttcaaccttttttgtatggctttcgctccaatctcgtgcagaaccatatttcatcttgggtttatgctgttctgtaagatctagcgccatgcagaggtcatttctgctgttccagaccccctacgtgacatttgctgtttttcctctttgttgccatggccacgggttggtttttacgaaagatactttgatatgtcaagatctgcgagcactttgaaaccccaacgcattttctatgtgttttgtgctgtttgatcgaccgattgatcgaggccgtgctagtactttgacacccgaaagcatctctcctttctgcagtatcttttctgttcttgtcgtctcttgggcttgtgcagtttaccatggtgaagagcgcttcatacacgatctgccgcgaggccagagcaaaagcttcccgtgctttttcttgcacagtgcatctccttcttttttgcctttttcgtttggacgtttctgcttcgtctccccatgtttctgttgtactgtcgcgcaccatgcatgttgattttctgatacgaagctagtactgctctgcagtttttgtgtagccttcctctttcgtgataaagaacgtggtcaaactgctctctgactctgttcgtctaaatctttttctcgcaggaaaattttcgttgcagatctcctttaccctcgtcctccgcatctgtttgctttacctgctgtagttgcgttcttcgtttgaatcaaattcttgtttccttcttttatcccatcgctcgtttagttaccttttctttttattgaactttagttcattggtgtagtaggcagtagtatgctttgcgttgtttgcggagtagcaattgaattgctctccggtctctgcagagcggcccgctgaacagatagctggctgcagcagctttaccagaatcggtcggttacgaacttacgattatacccttcgtcttgctttcatttactggtagcctgctagtcttttcttgttgcgcacgtaatcgtacccagtactgtacgcttagataaaatagacgggtctggccttaaattatttcgttgcgttttcgaattttgaattccggaagttaactttattttgtgctctgtttggacgcatgtgcaggtccagctcctcccgccgccgtcgtcagtgcccctcccccctccgccgcacctcgccgcaagcagccagcacgtacgaacaaccttttacacttcgcttgatctaattgctgctgctatactctcttactcgattctaaatctatgttttgctcattattaatatgttgatctgactcgtgtggcacgcgcgcgtgctttgatttcgcagacgaggcacctccgcctccgccgtcgactgagaagccgtccccgccgcctcagcaggacaacgtcaccgcccacggcaaggcaatccccacccatgcggccacatccccgctcgcgccggctgcttccatgatccacatgtccccaccgcccgcatgcaatccatgctccggctccgccgcttcctcagccgaggggcccctcctcatcgccgcgctcctcctcgtcatcaccgccatcatcgtcggcaccctcgacgataagtgatccaggagccgtccgccccctccgactcaccaacgtccgactatgatccagttgcagtagtggtcttgttctgtttcatgtttctcgccatttggttccgagatttctatatcgtgcctagtcgtagctgtagcagtcagtatgttcatgtgtccacaagatgtggtcgagtataacattgggtttcatgattcctctagcagatgaaacactatgtgatgtgatctgaatggatgcagttttgctaccttttctgctgctatgatatgcttatccatatgtttatctttcattcccttaatttgtgcggtttagcgttgtgttgccatgaatgcctcttgctctgctttgcgggttgcattttgtcttcgttctgctgtatatttgattctgaatttgcatgctgtgagtactaagtactgactacaatctctggatggttttgaaatttgaatgatgttataaaggagagctagctggggaattgcctcacctctaaactccaaaacacagagcagaagttggcctcaagatccaacttggtcactttgcatgtcggagcattgtagcaattctgcaataaacggagtagttctgttagcatgttgtttttacactgtcagtacaagtagaggtcgatgattaattatattccggttgtttgctgctggcttcccagttccctccaggtaggaaggaaccgtatccgggtagtagccagtagtagccaggaagctactagcagaacagtcttctggtgctctttttttggagtaacgtcttctcgcgatctttttcgagtaattcaaatccgggtataccgagccttgtatcagtgagagccgatagtcttaattatctccagcacaggcacaggaacaaccacgtttgtttttcagaatgcacagcaacattttttttaagagcatggcacagctactttttttttttttaaggaaacatggcacagctacatttttttttagaggaacatggcaca

SEQ ID NO: 45 - DNA, 684 bp, Brachypodium distachyon
atggagagatcccaccacctcctcctcgtgctcggcctcctcgccgcgctgctcccggcggccgcggctaccttcgggacgacgcagccggagcctggggccccatgcgagcccaccctcctcgccacccaggtctcgctcttctgcgcgccggacatgccgaccgcgcagtgctgcgagcctgtggtggcctccgtcgacctcgggggtggcgtcccctgcctctgccgtgtcgccgccgagccgcagctcgtcatggccggcctcaacgccacccacctcctcacgctctacacctcctgcggtggactccgccccggaggcgcccacctcgccgccgcctgtgaaggtccagctcctcccgccgccgtcgtcagtgcccctcccccctccgccgcacctcgccgcaagcagccagcacacgaggcacctccgcctccgccgtcgactgagaagccgtccccgccgcctcagcaggacaacgtcaccgcccacggcaaggcaatccccacccatgcggccacatccccgctcgcgccggctgcttccatgatccacatgtccccaccgcccgcatgcaatccatgctccggctccgccgcttcctcagccgaggggcccctcctcatcgccgcgctcctcctcgtcatcaccgccatcatcgtcggcaccctcgacgataag

SEQ ID NO: 46 - DNA, 951 bp, Triticum aestivum
tcgcgcgccgaccccgcgagagaccgtggtccgtccagtcgcagtagagtagagcgctcgtcgtctcgttccgtttcgtgcctgtcgccgttcgaggttcgtttctgcgtgcagtccggtcgaagaagccggtgggttttgagtactagtggtagtagtagcagcagctatcgtttctgtccgctcgtacgtgtttgcgtggtcgcggagaacaattaattgggtgtttgcgagtcctctggttaagatgaaccactgatgctatgtgatcgatcgatcggtatgatctgaatggaaatggatcaagttttgcgttctgctgatgatgtgatccatttggatctgtgtggggcaacagtttcgcttgcttttgctctgcgatgaacgaatgcttcttgcatgcatcttgtctttgcttaatttgaactgtagaacggatgcagtactgatttctgcttatgatgtgacgattcgtcgtacgcatatcatctcttcaaatttgtgtagcagctgtttgtagcttccattctgctatggacgaatgcctgtttttcacggagaaccgcgcgcggggaccgatgcggctttgtgttgccatgttgttttccacgccaggacaaaatagatggtgcggttttgatccccaatcccaccatcaccatgttccggagagccacatggaactcacgtcaagcggtcactttttgcagaatcactcttaccattttacccttttgttgaaacctctctcctcatccccaaaagttgatgcaacagtgctatgcgcgcccacccatgctttttcatatgattgtaaaatttggatcgattttatcttttgaaccctaagtccggtttacaatctgtttgcatgtttatgttccttgcggcgaggaccattaaacaagactactattggatatatttcgacaggctttgaaatccgaattc

SEQ ID NO: 47 - DNA, 1000 bp, Hordeum vulgare
tggccgacccccaaggcagcagagtacttgtcatctgattccgtttcatgcttgtcgccgtttgttgaggttcgtttctgcagtccgaacaagacggtggggttttgatcgggtacccagatttctatgtcgatcgcgcgtactagtactagtagttgcttagcagatgaacgaacattgggttttgggattcctctagctgatgaaccactgctattttccatgtgatcgatggatatgatctgaatggatggatgaagttttggtttctgatgctgatgatgtgctgcttcttcatttgcatgctcgatctattccttcaattttgtggagcaacagtttgtttagcttctgttctgctatgaataatgccgcttgcatcttgtcattgctgataatctgcttaatgcagacattgcttccgtcccaaacaatctgttgcttaccaggtaatgcatataatctgtacctcaccttcgcacaacaacagaagctaccctgctaaaaaaacacacacacacacacaaaaaaaacagaagctggtctcacacggaagccgcttcggggactgtttgcagctttttattgccattttgtttttcatgcaggtacaaatcgagggtgttgcttgatttgatcatggatgatcacttagagcaacatgtgtgttttgtctgtgttttattcgttgctcgtccatccaatttaaacttgaaatggatcgtgtgtggataaaagaagacgtgcgtcagtttgaatcgacgcgttgggttatattttgtgtctgtgacgaccgaaacgaagacaaaatatatcgtccggttagaattgctctaatgctagctttctctcctaccatcgcattccgtggtaggaaaaagtactagaaccacaggaaactggaacgcaagaaaagcatatctaccgttggccgttgatcttgtttcacattcggtatggctccggtcatattgttggagattcacattcatgcacgcaa